European Patent Specification EP 3 630 197 B1, published August 16, 2023. Title: Method of selecting genetically modified hematopoietic stem cells. Applicant: COMMISSARIAT A L'ENERGIE ATOMIQUE ET AUX ENERGIES ALTERNATIVES INSERM (Institut National de la Santé et de la Recherche Médicale). The sequence listing filed with the application follows.

SEQUENCE LISTING (7 sequences)

SEQ ID NO: 1 - DNA, 1840 bp, artificial sequence
  synthetic polynucleotide
ggctccggtgcccgtcagtgggcagagcgcacatcgcccacagtccccgagaagttggggggaggggtcggcaattgaaccggtgcctagagaaggtggcgcggggtaaactgggaaagtgatgtcgtgtactggctccgcctttttcccgagggtgggggagaaccgtatataagtgcagtagtcgccgtgaacgttctttttcgcaacgggtttgccgccagaacacaggctagccaccatgacggagtataagccgactgtcaggctggccacaagggacgatgtgcccagggccgtcagaactctggcagcagctttcgcagactacccggcgaccagacatacggtggaccctgacagacatattgagcgcgtgacggagttgcaagaacttttcttgacccgagtcggactcgacatcgggaaggtgtgggtggcggatgatggagcagccgtcgcggtatggacaacgcccgaatcagtcgaggctggagcggtctttgcggaaatcggccctagaatggcggaactttccgggagccggctggcggcacagcagcagatggagggactgttggcacctcaccgcccgaaagagccggcctggttcctggcgacagtcggtgtatcacccgaccaccaggggaaaggtctgggttccgccgtggtgttgcctggagtggaggcagccgagagagcaggggtcccagcgtttttggaaaccagcgcgccacggaacctcccattctacgagcggctcggattcaccgtaacggccgacgtagaagtaccggaaggacctcggacttggtgcatgaccagaaagcccggtgcggggtcgatgcccactcttttgcgggtatacattgatgggccgcatggaatgggaaagaccacaacaacgcagctccttgtcgcgctgggtagccgggacgacattgtctatgtgcccgagccgatgacttactggagggtattgggtgcgagcgaaacgattgccaacatctacactacacagcaccgcttggatcagggcgagatttcagcgggtgatgccgcagtggtgatgacgtcggcgcagatcacaatgggaatgccgtatgcggtgacggatgcggtacttgcgcctcacatcgggggagaggcgggctcctcgcatgcccctcccccagcactcacgctcatctttgatcgccatccaatcgccgctctcctttgctacccggctgcccgatacctgatgggttcgatgacgccccaagctgtattggcgtttgtcgcgttgatcccgcccacgctgccagggaccaatatcgtcttgggggcattgcccgaggataggcacattgacagactggccaaaaggcagaggcccggagagcgattggacttggccatgctcgcggccattagacgggtgtatggattgctcgcaaatacggtgcgctatctgcagtgtggtggatcatggcgcgaggactggggtcagctttcgggcactgcagtacccccgcaaggtgcagaaccccagagcaacgcgggaccccgaccacacatcggagacacgctgttcacattgtttagagcccccgaacttctcgcgcctaatggggacctctacaacgtattcgcatgggcgcttgatgtcttggcgaaaaggcttaggtcgatgcacgtgttcatcttggattatgaccagtcgccggcaggatgcagggatgctctgctgcaactgacgtcggggatggtgcagactcatgtgaccacccccggatcaattcctactatctgtgatctggcgcgcacctttgcgcgagaaatgggggaagccaattga

SEQ ID NO: 2 - DNA, 20 bp, artificial sequence
  synthetic oligonucleotide
tgtgtgcccgtctgttgtgt

SEQ ID NO: 3 - DNA, 19 bp, artificial sequence
  synthetic oligonucleotide
cgagtcctgcgtcgagaga

SEQ ID NO: 4 - DNA, 20 bp, artificial sequence
  synthetic oligonucleotide
cagtggcgcccgaacaggga

SEQ ID NO: 5 - DNA, 25 bp, artificial sequence
  synthetic oligonucleotide
tattagcaccatccataggaggctt

SEQ ID NO: 6 - DNA, 22 bp, artificial sequence
  synthetic oligonucleotide
gttagggaaagtggagcggaag

SEQ ID NO: 7 - DNA, 25 bp, artificial sequence
  synthetic oligonucleotide
taacgcgtccaccaaggatgcgaat